European Patent Specification EP 3 168 766 B1, published August 16, 2023. Title: MELTING CURVE ANALYSIS WITH EXPONENTIAL BACKGROUND SUBTRACTION. Applicant: University of Utah Research Foundation Palais, Robert A. Wittwer, Carl T. Application US 12/067,642. The sequence listing filed with the application follows.

SEQUENCE LISTING (9 sequences)

SEQ ID NO: 1 - DNA, 100 bp, Homo sapiens
ctgaaaggttacttcaaggacaaaatacctgtattcctcgcctgtccagggatctgctcttacagattagaagtagtcctattagcccagaggcgatgtc

SEQ ID NO: 2 - DNA, 21 bp, Homo sapiens
ctgaaaggttacttcaaggac

SEQ ID NO: 3 - DNA, 15 bp, Homo sapiens
gacatcgcctctggg

SEQ ID NO: 4 - DNA, 22 bp, Homo sapiens
tggacataaggagcggacaggt

SEQ ID NO: 5 - DNA, 10 bp, Homo sapiens
tcttggagaa

SEQ ID NO: 6 - DNA, 10 bp, Homo sapiens
aggtcaacga

SEQ ID NO: 7 - DNA, 10 bp, Homo sapiens
ttctcagttt

SEQ ID NO: 8 - DNA, 11 bp, Homo sapiens
tatcatctttg

SEQ ID NO: 9 - DNA, 45 bp, Homo sapiens
ccatggtgcacctgactcctgaggagaagtctgccgttactgccc